European Patent Application EP 4 715 062 A1, published March 25, 2026. Title: Biomarkers for determining stress levels. Applicant: National Institute of Advanced Industrial Science and Technology. The sequence listing filed with the application follows.

SEQUENCE LISTING (122 sequences)

SEQ ID NO: 1 - DNA, 64 bp, synthetic construct
  source 1..64: mol_type = other DNA
cgacgctcttccgatctctgtcgccctgaacaacggcaatggcagtcagatcggaagagcacac

SEQ ID NO: 2 - DNA, 62 bp, synthetic construct
  source 1..62: mol_type = other DNA
cgacgctcttccgatctctgtgccgctagccagggttggactgtcagatcggaagagcacac

SEQ ID NO: 3 - DNA, 64 bp, synthetic construct
  source 1..64: mol_type = other DNA
cgacgctcttccgatctctggcactcgttgctgggtctggggacgtcagatcggaagagcacac

SEQ ID NO: 4 - DNA, 63 bp, synthetic construct
  source 1..63: mol_type = other DNA
cgacgctcttccgatctctgacagctactcgtgcgggaaagcagtcagatcggaagagcacac

SEQ ID NO: 5 - DNA, 64 bp, synthetic construct
  source 1..64: mol_type = other DNA
cgacgctcttccgatctctgggtctggggtcaactccgtggcgtgtcagatcggaagagcacac

SEQ ID NO: 6 - DNA, 64 bp, synthetic construct
  source 1..64: mol_type = other DNA
cgacgctcttccgatctctgggcgaagtctcaatcggcgatcgggtcagatcggaagagcacac

SEQ ID NO: 7 - DNA, 64 bp, synthetic construct
  source 1..64: mol_type = other DNA
cgacgctcttccgatctctgtgtggcagccattcgttcctccgcgtcagatcggaagagcacac

SEQ ID NO: 8 - DNA, 64 bp, synthetic construct
  source 1..64: mol_type = other DNA
cgacgctcttccgatctctgacccaagcgatctgactgtccaccgtcagatcggaagagcacac

SEQ ID NO: 9 - DNA, 62 bp, synthetic construct
  source 1..62: mol_type = other DNA
cgacgctcttccgatctctgtcctccaaggagccgccacaccgtcagatcggaagagcacac

SEQ ID NO: 10 - DNA, 62 bp, synthetic construct
  source 1..62: mol_type = other DNA
cgacgctcttccgatctctgcgtgctgacgatgggtggcagtgtcagatcggaagagcacac

SEQ ID NO: 11 - DNA, 62 bp, synthetic construct
  source 1..62: mol_type = other DNA
cgacgctcttccgatctctgagcggctggtgtgtaggggccagtcagatcggaagagcacac

SEQ ID NO: 12 - DNA, 63 bp, synthetic construct
  source 1..63: mol_type = other DNA
cgacgctcttccgatctctgcgtatggcggtagcggtggtagcgtcagatcggaagagcacac

SEQ ID NO: 13 - DNA, 64 bp, synthetic construct
  source 1..64: mol_type = other DNA
cgacgctcttccgatctctgtgggagtccacagggaagcagtgtgtcagatcggaagagcacac

SEQ ID NO: 14 - DNA, 64 bp, synthetic construct
  source 1..64: mol_type = other DNA
cgacgctcttccgatctctggggtggcaatggaggcagtgcacagtcagatcggaagagcacac

SEQ ID NO: 15 - DNA, 64 bp, synthetic construct
  source 1..64: mol_type = other DNA
cgacgctcttccgatctctgtggtgaacggcctgcaagtcgtgtgtcagatcggaagagcacac

SEQ ID NO: 16 - DNA, 63 bp, synthetic construct
  source 1..63: mol_type = other DNA
cgacgctcttccgatctctggtgggaatggtggctcagcgttcgtcagatcggaagagcacac

SEQ ID NO: 17 - DNA, 62 bp, synthetic construct
  source 1..62: mol_type = other DNA
cgacgctcttccgatctctgggcggcaacaatcccattgcgtgtcagatcggaagagcacac

SEQ ID NO: 18 - DNA, 61 bp, synthetic construct
  source 1..61: mol_type = other DNA
cgacgctcttccgatctctgtgcgaatgcagccaacacgcagtcagatcggaagagcacac

SEQ ID NO: 19 - DNA, 62 bp, synthetic construct
  source 1..62: mol_type = other DNA
cgacgctcttccgatctctgactgatgcgcgtttagccccgagtcagatcggaagagcacac

SEQ ID NO: 20 - DNA, 64 bp, synthetic construct
  source 1..64: mol_type = other DNA
cgacgctcttccgatctctgactggcagaaaggtcgcgaagagcgtcagatcggaagagcacac

SEQ ID NO: 21 - DNA, 64 bp, synthetic construct
  source 1..64: mol_type = other DNA
cgacgctcttccgatctctgtccgtccattcgcgtctacaccgcgtcagatcggaagagcacac

SEQ ID NO: 22 - DNA, 63 bp, synthetic construct
  source 1..63: mol_type = other DNA
cgacgctcttccgatctctgtggaaagtgggtcgctcagtggggtcagatcggaagagcacac

SEQ ID NO: 23 - DNA, 64 bp, synthetic construct
  source 1..64: mol_type = other DNA
cgacgctcttccgatctctgtggcaagtctgctgggatcatggcgtcagatcggaagagcacac

SEQ ID NO: 24 - DNA, 62 bp, synthetic construct
  source 1..62: mol_type = other DNA
cgacgctcttccgatctctgatgttgcgaaagcgggcatacggtcagatcggaagagcacac

SEQ ID NO: 25 - DNA, 61 bp, synthetic construct
  source 1..61: mol_type = other DNA
cgacgctcttccgatctctgagtgacgacggtggcttgccagtcagatcggaagagcacac

SEQ ID NO: 26 - DNA, 64 bp, synthetic construct
  source 1..64: mol_type = other DNA
cgacgctcttccgatctctggccggcgaaatcacatgtgtttgcgtcagatcggaagagcacac

SEQ ID NO: 27 - DNA, 61 bp, synthetic construct
  source 1..61: mol_type = other DNA
cgacgctcttccgatctctgctcgccacgcatccactggtggtcagatcggaagagcacac

SEQ ID NO: 28 - DNA, 64 bp, synthetic construct
  source 1..64: mol_type = other DNA
cgacgctcttccgatctctgggactccgattgtaggctggcagtgtcagatcggaagagcacac

SEQ ID NO: 29 - DNA, 64 bp, synthetic construct
  source 1..64: mol_type = other DNA
cgacgctcttccgatctctgtgccacgatgcgttctgtggagccgtcagatcggaagagcacac

SEQ ID NO: 30 - DNA, 63 bp, synthetic construct
  source 1..63: mol_type = other DNA
cgacgctcttccgatctctgtggcctttcacttcaacccacgcgtcagatcggaagagcacac

SEQ ID NO: 31 - DNA, 63 bp, synthetic construct
  source 1..63: mol_type = other DNA
cgacgctcttccgatctctgcgcttgcttgggtttgccagtcggtcagatcggaagagcacac

SEQ ID NO: 32 - DNA, 64 bp, synthetic construct
  source 1..64: mol_type = other DNA
cgacgctcttccgatctctggcgagtccgtattgccgtccaccggtcagatcggaagagcacac

SEQ ID NO: 33 - DNA, 64 bp, synthetic construct
  source 1..64: mol_type = other DNA
cgacgctcttccgatctctgtggtactcgcaccttggaaaccgtgtcagatcggaagagcacac

SEQ ID NO: 34 - DNA, 62 bp, synthetic construct
  source 1..62: mol_type = other DNA
cgacgctcttccgatctctgtggtgcagctctggttggctcagtcagatcggaagagcacac

SEQ ID NO: 35 - DNA, 64 bp, synthetic construct
  source 1..64: mol_type = other DNA
cgacgctcttccgatctctggccaaagctgcagatggccttgccgtcagatcggaagagcacac

SEQ ID NO: 36 - DNA, 62 bp, synthetic construct
  source 1..62: mol_type = other DNA
cgacgctcttccgatctctgtgggtggctctgggacctcagggtcagatcggaagagcacac

SEQ ID NO: 37 - DNA, 64 bp, synthetic construct
  source 1..64: mol_type = other DNA
cgacgctcttccgatctctgtccaaccgcgcaacatcacgaccagtcagatcggaagagcacac

SEQ ID NO: 38 - DNA, 61 bp, synthetic construct
  source 1..61: mol_type = other DNA
cgacgctcttccgatctctggccgtgttggtcgtgcttcgggtcagatcggaagagcacac

SEQ ID NO: 39 - DNA, 62 bp, synthetic construct
  source 1..62: mol_type = other DNA
cgacgctcttccgatctctgagcgttcttcttggcacccgctgtcagatcggaagagcacac

SEQ ID NO: 40 - DNA, 61 bp, synthetic construct
  source 1..61: mol_type = other DNA
cgacgctcttccgatctctggcttggcaagcgttcctggctgtcagatcggaagagcacac

SEQ ID NO: 41 - DNA, 62 bp, synthetic construct
  source 1..62: mol_type = other DNA
cgacgctcttccgatctctgacgagcgactcaaggacaagtggtcagatcggaagagcacac

SEQ ID NO: 42 - DNA, 22 bp, synthetic construct
  source 1..22: mol_type = other DNA
tcgccctgaacaacggcaatgg

SEQ ID NO: 43 - DNA, 22 bp, synthetic construct
  source 1..22: mol_type = other DNA
tgccgctagccagggttggact

SEQ ID NO: 44 - DNA, 22 bp, synthetic construct
  source 1..22: mol_type = other DNA
gcactcgttgctgggtctgggg

SEQ ID NO: 45 - DNA, 22 bp, synthetic construct
  source 1..22: mol_type = other DNA
acagctactcgtgcgggaaagc

SEQ ID NO: 46 - DNA, 22 bp, synthetic construct
  source 1..22: mol_type = other DNA
ggtctggggtcaactccgtggc

SEQ ID NO: 47 - DNA, 22 bp, synthetic construct
  source 1..22: mol_type = other DNA
ggcgaagtctcaatcggcgatc

SEQ ID NO: 48 - DNA, 22 bp, synthetic construct
  source 1..22: mol_type = other DNA
tgtggcagccattcgttcctcc

SEQ ID NO: 49 - DNA, 22 bp, synthetic construct
  source 1..22: mol_type = other DNA
acccaagcgatctgactgtcca

SEQ ID NO: 50 - DNA, 22 bp, synthetic construct
  source 1..22: mol_type = other DNA
tcctccaaggagccgccacacc

SEQ ID NO: 51 - DNA, 22 bp, synthetic construct
  source 1..22: mol_type = other DNA
cgtgctgacgatgggtggcagt

SEQ ID NO: 52 - DNA, 22 bp, synthetic construct
  source 1..22: mol_type = other DNA
agcggctggtgtgtaggggcca

SEQ ID NO: 53 - DNA, 22 bp, synthetic construct
  source 1..22: mol_type = other DNA
cgtatggcggtagcggtggtag

SEQ ID NO: 54 - DNA, 22 bp, synthetic construct
  source 1..22: mol_type = other DNA
tgggagtccacagggaagcagt

SEQ ID NO: 55 - DNA, 22 bp, synthetic construct
  source 1..22: mol_type = other DNA
gggtggcaatggaggcagtgca

SEQ ID NO: 56 - DNA, 22 bp, synthetic construct
  source 1..22: mol_type = other DNA
tggtgaacggcctgcaagtcgt

SEQ ID NO: 57 - DNA, 22 bp, synthetic construct
  source 1..22: mol_type = other DNA
gtgggaatggtggctcagcgtt

SEQ ID NO: 58 - DNA, 22 bp, synthetic construct
  source 1..22: mol_type = other DNA
ggcggcaacaatcccattgcgt

SEQ ID NO: 59 - DNA, 21 bp, synthetic construct
  source 1..21: mol_type = other DNA
tgcgaatgcagccaacacgca

SEQ ID NO: 60 - DNA, 22 bp, synthetic construct
  source 1..22: mol_type = other DNA
actgatgcgcgtttagccccga

SEQ ID NO: 61 - DNA, 22 bp, synthetic construct
  source 1..22: mol_type = other DNA
actggcagaaaggtcgcgaaga

SEQ ID NO: 62 - DNA, 22 bp, synthetic construct
  source 1..22: mol_type = other DNA
tccgtccattcgcgtctacacc

SEQ ID NO: 63 - DNA, 22 bp, synthetic construct
  source 1..22: mol_type = other DNA
tggaaagtgggtcgctcagtgg

SEQ ID NO: 64 - DNA, 22 bp, synthetic construct
  source 1..22: mol_type = other DNA
tggcaagtctgctgggatcatg

SEQ ID NO: 65 - DNA, 22 bp, synthetic construct
  source 1..22: mol_type = other DNA
atgttgcgaaagcgggcatacg

SEQ ID NO: 66 - DNA, 21 bp, synthetic construct
  source 1..21: mol_type = other DNA
agtgacgacggtggcttgcca

SEQ ID NO: 67 - DNA, 22 bp, synthetic construct
  source 1..22: mol_type = other DNA
gccggcgaaatcacatgtgttt

SEQ ID NO: 68 - DNA, 21 bp, synthetic construct
  source 1..21: mol_type = other DNA
ctcgccacgcatccactggtg

SEQ ID NO: 69 - DNA, 22 bp, synthetic construct
  source 1..22: mol_type = other DNA
ggactccgattgtaggctggca

SEQ ID NO: 70 - DNA, 22 bp, synthetic construct
  source 1..22: mol_type = other DNA
tgccacgatgcgttctgtggag

SEQ ID NO: 71 - DNA, 22 bp, synthetic construct
  source 1..22: mol_type = other DNA
tggcctttcacttcaacccacg

SEQ ID NO: 72 - DNA, 22 bp, synthetic construct
  source 1..22: mol_type = other DNA
cgcttgcttgggtttgccagtc

SEQ ID NO: 73 - DNA, 22 bp, synthetic construct
  source 1..22: mol_type = other DNA
gcgagtccgtattgccgtccac

SEQ ID NO: 74 - DNA, 22 bp, synthetic construct
  source 1..22: mol_type = other DNA
tggtactcgcaccttggaaacc

SEQ ID NO: 75 - DNA, 22 bp, synthetic construct
  source 1..22: mol_type = other DNA
tggtgcagctctggttggctca

SEQ ID NO: 76 - DNA, 22 bp, synthetic construct
  source 1..22: mol_type = other DNA
gccaaagctgcagatggccttg

SEQ ID NO: 77 - DNA, 22 bp, synthetic construct
  source 1..22: mol_type = other DNA
tgggtggctctgggacctcagg

SEQ ID NO: 78 - DNA, 22 bp, synthetic construct
  source 1..22: mol_type = other DNA
tccaaccgcgcaacatcacgac

SEQ ID NO: 79 - DNA, 21 bp, synthetic construct
  source 1..21: mol_type = other DNA
gccgtgttggtcgtgcttcgg

SEQ ID NO: 80 - DNA, 22 bp, synthetic construct
  source 1..22: mol_type = other DNA
agcgttcttcttggcacccgct

SEQ ID NO: 81 - DNA, 22 bp, synthetic construct
  source 1..22: mol_type = other DNA
cgctcttccgatctctggcttg

SEQ ID NO: 82 - DNA, 22 bp, synthetic construct
  source 1..22: mol_type = other DNA
acgagcgactcaaggacaagtg

SEQ ID NO: 83 - DNA, 46 bp, synthetic construct
  source 1..46: mol_type = other DNA
tcgtcgcagcgtcagatgtgtataagacagcctacggnggcwgcag

SEQ ID NO: 84 - DNA, 55 bp, synthetic construct
  source 1..55: mol_type = other DNA
gtctcgtgggctcggagatgtgtataagagacaggactachvgggtatctaatcc

SEQ ID NO: 85 - DNA, 68 bp, synthetic construct
  source 1..68: mol_type = other DNA
caagcagaagacggcatacgagatnnnnnnnngtgactggagttcagacgtgtgctcttccgatctga

SEQ ID NO: 86 - DNA, 73 bp, synthetic construct
  source 1..73: mol_type = other DNA
aatgatacggcgaccaccgagatctacacnnnnnnnnacactctttccctacacgacgctcttccgatctctg

SEQ ID NO: 87-122 - skipped (36 entries)